European Patent Specification EP 3 294 353 B1, published October 25, 2023. Title: Haemostatic Compositions. Applicant: Haemostatix Limited. The sequence listing filed with the application follows.

SEQUENCE LISTING (17 sequences)

SEQ ID NO: 1 - protein, 4 aa, Homo sapiens
GPRP

SEQ ID NO: 2 - protein, 4 aa, Homo sapiens
GPRV

SEQ ID NO: 3 - protein, 7 aa, Homo sapiens
GPRPFPA

SEQ ID NO: 4 - protein, 7 aa, Homo sapiens
GPRVVAA

SEQ ID NO: 5 - protein, 8 aa, Homo sapiens
GPRPVVER

SEQ ID NO: 6 - protein, 6 aa, Homo sapiens
GPRPAA

SEQ ID NO: 7 - protein, 7 aa, Homo sapiens
GPRPPEC

SEQ ID NO: 8 - protein, 7 aa, Homo sapiens
GPRPPER

SEQ ID NO: 9 - protein, 6 aa, Homo sapiens
GPSPAA

SEQ ID NO: 10 - protein, 4 aa, Homo sapiens
GHRP

SEQ ID NO: 11 - protein, 5 aa, Homo sapiens
GHRPY

SEQ ID NO: 12 - protein, 5 aa, Homo sapiens
GHRPL

SEQ ID NO: 13 - protein, 5 aa, Homo sapiens
  MISC_FEATURE (5)..(5): Carboxy-terminal end comprises an amide group
GHRPY

SEQ ID NO: 14 - protein, 7 aa, Homo sapiens
  MISC_FEATURE (7)..(7): Carboxy-terminal end may comprise an amide group
APFPRPG

SEQ ID NO: 15 - protein, 4 aa, Homo sapiens
  MISC_FEATURE (2)..(2): Pro or His
  MISC_FEATURE (4)..(4): Any amino acid
GXRX

SEQ ID NO: 16 - protein, 5 aa, Homo sapiens
  misc_feature (5)..(5): Carboxy-terminal end comprises an amide group
YPRHG

SEQ ID NO: 17 - protein, 5 aa, Homo sapiens
GPRPG